European Patent Specification EP 4 274 565 B1, published April 22, 2026. Title: Soy Isoflavones for Asthma Prevention. Applicant: University of South Florida. The sequence listing filed with the application follows.

SEQUENCE LISTING (4 sequences)

SEQ ID NO: 1 - DNA, 17 bp, Homo sapiens
gtctggacacgtggggg

SEQ ID NO: 2 - DNA, 17 bp, Homo sapiens
gtctggacacgtgggga

SEQ ID NO: 3 - DNA, 25 bp, Homo sapiens
tgcagccagccacgtgattgtctag

SEQ ID NO: 4 - DNA, 26 bp, Homo sapiens
aagcttttaccatggtaacccctggt